European Patent Application EP 4 628 598 A1, published October 8, 2025. Title: DNA methylation marker for determination of T-status of cancer. Applicant: Siemens Healthcare Diagnostics Products GmbH. Application EP. The sequence listing filed with the application follows.

SEQUENCE LISTING (1 sequence)

SEQ ID NO: 1 - DNA, 82 bp, Homo sapiens
  source 1..82: mol_type = genomic DNA
ggcaggggctgtgcgcggctctctcccctaaagcgaggttcgtgctcatctctagcccccgccgctctcgtgggccacgtcc